European Patent Application EP 4 509 601 A1, published February 19, 2025. Title: 一种凝血因子X激活酶及其应用. Applicant: 北京三诺佳邑生物技术有限责任公司. The sequence listing filed with the application follows.

SEQUENCE LISTING (15 sequences)

SEQ ID NO: 1 - DNA, 31 bp, synthetic construct
  source 1..31: mol_type = other DNA
atgatgcaagttctcttagtaactataagct

SEQ ID NO: 2 - DNA, 26 bp, synthetic construct
  source 1..26: mol_type = other DNA
tcaaatctgagagaagccagtggttg

SEQ ID NO: 3 - DNA, 26 bp, synthetic construct
  source 1..26: mol_type = other DNA
atggggcgattcatctccgtcagctt

SEQ ID NO: 4 - DNA, 30 bp, synthetic construct
  source 1..30: mol_type = other DNA
ggatcttaacactctggtggcaccttgcag

SEQ ID NO: 5 - DNA, 28 bp, synthetic construct
  source 1..28: mol_type = other DNA
aggaaggaagaccatggggcgattcatc

SEQ ID NO: 6 - DNA, 28 bp, synthetic construct
  source 1..28: mol_type = other DNA
cctagaacttgcacacgacaggtgctat

SEQ ID NO: 7 - protein, 619 aa
MMQVLLVTISLAVFPYQGSSIILESGNVNDYEVVYPQKVTALPKGAVQQPEQKYEDTMQYEFEVNGEPVVLHLEKNKILFSEDYSETHYSPDGREITTNPPVEDHCYYHGRIQNDAHSSASISACNGLKGHFKLRGEMYFIEPLKLSNNEAHAVYKYENIEKEDETPKMCGVTQTNWESDEPIKKASQLVATSAQFNKAFIELIIIVDHSMAKKCNSTATNTKIYEIVNSANEIFNPLNIHVTLIGVEFWCDRDLINVTSSADETLDSFGEWRASDLMTRKSHDNALLFTDMRFDLNTLGITFLAGMCQAYRSVGIVQVQGNRNFKTAVIMAHELSHNLGMYHDGKNCICNDSSCVMSPVLSDQPSKLFSNCSIHDYQRYLTRYKPKCILYPPLRKDIVSPPVCGNEIWEEGEECDCGSPADCQNPCCDAATCKLKPGAECGNGLCCYQCKIKTAGTVCRRARNECDVPEHCTGQSAECPRDQLQQNGQPCQNNRGYCYNGDCPIMRNQCISLFGSRANVAKDSCFQENLKGSYYGYCRKENGRKIPCAPQDVKCGRLFCLNNSPGNKNPCNMHYSCMDQHKGMVDPGTKCEDGKVCNNKRQCVDVNTAYQSTTGFSQI

SEQ ID NO: 8 - protein, 431 aa, synthetic construct
LVATSAQFNKAFIELIIIVDHSMAKKCNSTATNTKIYEIVNSANEIFNPLNIHVTLIGVEFWCDRDLINVTSSADETLDSFGEWRASDLMTRKSHDNALLFTDMRFDLNTLGITFLAGMCQAYRSVGIVQVQGNRNFKTAVIMAHELSHNLGMYHDGKNCICNDSSCVMSPVLSDQPSKLFSNCSIHDYQRYLTRYKPKCILYPPLRKDIVSPPVCGNEIWEEGEECDCGSPADCQNPCCDAATCKLKPGAECGNGLCCYQCKIKTAGTVCRRARNECDVPEHCTGQSAECPRDQLQQNGQPCQNNRGYCYNGDCPIMRNQCISLFGSRANVAKDSCFQENLKGSYYGYCRKENGRKIPCAPQDVKCGRLFCLNNSPGNKNPCNMHYSCMDQHKGMVDPGTKCEDGKVCNNKRQCVDVNTAYQSTTGFSQI

SEQ ID NO: 9 - protein, 158 aa, synthetic construct
MGRFISVSFGLLVVFLSLSGTGAGLDCPPDSSLYRYFCYRVFKEHKTWEAAERFCMEHPNNGHLVSVESMEEAEFVAKLLSNITEKFITHFWIGLMIKDKEQECSSEWSDGSSVSYDNLDKREFRKCFVLEKESGYRMWFNRNCEERYLFVCKVPPEC

SEQ ID NO: 10 - protein, 135 aa, synthetic construct
GLDCPPDSSLYRYFCYRVFKEHKTWEAAERFCMEHPNNGHLVSVESMEEAEFVAKLLSNITEKFITHFWIGLMIKDKEQECSSEWSDGSSVSYDNLDKREFRKCFVLEKESGYRMWFNRNCEERYLFVCKVPPEC

SEQ ID NO: 11 - protein, 146 aa, synthetic construct
MGRFISVSFGCLVVFLSLSGTEAVLDCPSGWLSYEQHCYKGFNDLKNWTDAEKFCTEQKKGSHLVSLHSREEEEFVVNLISENLEYPATWIGLGNMWKDCRMEWSDRGNVKYKALAEESYCLIMITHEKEWKSMTCNFIAPVVCKF

SEQ ID NO: 12 - protein, 123 aa, synthetic construct
VLDCPSGWLSYEQHCYKGFNDLKNWTDAEKFCTEQKKGSHLVSLHSREEEEFVVNLISENLEYPATWIGLGNMWKDCRMEWSDRGNVKYKALAEESYCLIMITHEKEWKSMTCNFIAPVVCKF

SEQ ID NO: 13 - protein, 35 aa, synthetic construct
LVATSAQFNKAFIELIIIVDHSMAKKCNSTATNTK

SEQ ID NO: 14 - protein, 63 aa, synthetic construct
GLDCPPDSSLYRYFCYRVFKEHKTWEAAERFCMEHPNNGHLVSVESMEEAEFVAKLLSNITEK

SEQ ID NO: 15 - protein, 47 aa, synthetic construct
VLDCPSGWLSYEQHCYKGFNDLKNWTDAEKFCTEQKKGSHLVSLHSR